European Patent Specification EP 3 898 985 B1, published February 8, 2023. Title: Tandem Protein Expression. Applicant: Novozymes A/S. The sequence listing filed with the application follows.

SEQUENCE LISTING (11 sequences)

SEQ ID NO: 1 - DNA, 105 bp, Artificial Sequence
  DNA sequence of CPP used as signal peptide
atgaagttcttcaccaccatcctcagcaccgccagccttgttgctgctctccccgccgctgttgactcgaaccataccccggccgctcctgaacttgttgcccgg

SEQ ID NO: 2 - protein, 35 aa, Artificial Sequence
  Amino acid sequence of CPP used as signal peptide
MKFFTTILSTASLVAALPAAVDSNHTPAAPELVAR

SEQ ID NO: 3 - DNA, 1059 bp, Valsaria rubricosa
atgaagtccgcttcgatcttactcagggtagctgccctcctcctccctgctgtatctgcactgccacttgaaagaagaggtatggacgaactatcctagcgatcagtgtgtctattttgcctaacctagcaaagctatatccgcggatctcctggcaaccttcagcctcttcgagcagttcgcagccgcagcatattgtccggataacaacgacagtcccgacaccaagcttacttgctctgtcggaaactgcccgcttgtcgaagctgacacgaccagcacggtcactgaattcgaaaagtacatcttacacgaccccgttcacctacagacaaagtcccagctaacgtccacctctatctctgtccctttagctcgctcgaaaccgacgtcactggctacgtcgcgactgacagcacacgagagctcatcgttgtggcattccgcgggagttcctcgatccggaactggatcgccgacatcgactttcccttcaccgacaccgacctctgcgatggctgccaggcagcctcgggcttctggacgtcctggacggaggcacggacaggggtgctggcggcggtggcgagcgctgccgcggccaacccgtcctataccgttgccgtgacgggccacagcctcggcggggccgtggccgcgctggccgctggcgccctccggaacgcgggctacacggtcgcgctatacagcttcggagcgcctcgcgtgggtgacgagaccctcagcgagtacatcactgcgcaggcgggtggaaactaccgcatcacgcacctcaacgacccagtgccgaagctgcccccgctgctcctggggtatcgccacatcagcccggaatactacatcagcagcgggaacaacgtgaccgtgacggcggatgacgtggaggagtacaccggcacgatcaacctgagtgggaacacgggcgatctgacgttcgacacggatgcgcacagttggtacttcaacgagatcggggcatgcgatgatggtgaggctttggagtggaagaagcggggggtagaagttcagtgggtttaa

SEQ ID NO: 4 - DNA, 930 bp, Artificial Sequence
  cDNA of DNA sequence of LipVR gene
  CDS (1)..(927)
  sig_peptide (1)..(60)
  mat_peptide (61)..(927)
atgaagtccgcttcgatcttactcagggtagctgccctcctcctccctgctgtatctgcactgccacttgaaagaagagctatatccgcggatctcctggcaaccttcagcctcttcgagcagttcgcagccgcagcatattgtccggataacaacgacagtcccgacaccaagcttacttgctctgtcggaaactgcccgcttgtcgaagctgacacgaccagcacggtcactgaattcgaaaactcgctcgaaaccgacgtcactggctacgtcgcgactgacagcacacgagagctcatcgttgtggcattccgcgggagttcctcgatccggaactggatcgccgacatcgactttcccttcaccgacaccgacctctgcgatggctgccaggcagcctcgggcttctggacgtcctggacggaggcacggacaggggtgctggcggcggtggcgagcgctgccgcggccaacccgtcctataccgttgccgtgacgggccacagcctcggcggggccgtggccgcgctggccgctggcgccctccggaacgcgggctacacggtcgcgctatacagcttcggagcgcctcgcgtgggtgacgagaccctcagcgagtacatcactgcgcaggcgggtggaaactaccgcatcacgcacctcaacgacccagtgccgaagctgcccccgctgctcctggggtatcgccacatcagcccggaatactacatcagcagcgggaacaacgtgaccgtgacggcggatgacgtggaggagtacaccggcacgatcaacctgagtgggaacacgggcgatctgacgttcgacacggatgcgcacagttggtacttcaacgagatcggggcatgcgatgatggtgaggctttggagtggaagaagcggggggtagaagttcagtgggtttaa

SEQ ID NO: 5 - protein, 309 aa, Artificial Sequence
  Synthetic Construct
MKSASILLRVAALLLPAVSALPLERRAISADLLATFSLFEQFAAAAYCPDNNDSPDTKLTCSVGNCPLVEADTTSTVTEFENSLETDVTGYVATDSTRELIVVAFRGSSSIRNWIADIDFPFTDTDLCDGCQAASGFWTSWTEARTGVLAAVASAAAANPSYTVAVTGHSLGGAVAALAAGALRNAGYTVALYSFGAPRVGDETLSEYITAQAGGNYRITHLNDPVPKLPPLLLGYRHISPEYYISSGNNVTVTADDVEEYTGTINLSGNTGDLTFDTDAHSWYFNEIGACDDGEALEWKKRGVEVQWV

SEQ ID NO: 6 - protein, 289 aa, Valsaria rubricosa
LPLERRAISADLLATFSLFEQFAAAAYCPDNNDSPDTKLTCSVGNCPLVEADTTSTVTEFENSLETDVTGYVATDSTRELIVVAFRGSSSIRNWIADIDFPFTDTDLCDGCQAASGFWTSWTEARTGVLAAVASAAAANPSYTVAVTGHSLGGAVAALAAGALRNAGYTVALYSFGAPRVGDETLSEYITAQAGGNYRITHLNDPVPKLPPLLLGYRHISPEYYISSGNNVTVTADDVEEYTGTINLSGNTGDLTFDTDAHSWYFNEIGACDDGEALEWKKRGVEVQWV

SEQ ID NO: 7 - DNA, 41 bp, Artificial Sequence
  Primer lipVR-A
tacacaactgggggccaccatgaagtccgcttcgatcttac

SEQ ID NO: 8 - DNA, 38 bp, Artificial Sequence
  Primer lipVR-B
gtgtcagtcaccgcgttaaacccactgaacttctaccc

SEQ ID NO: 9 - DNA, 2028 bp, Artificial Sequence
  DNA sequence of lipVR-tandem
atgaagttcttcaccaccatcctcagcaccgccagccttgttgctgctctccccgccgctgttgactcgaaccataccccggccgctcctgaacttgttgcccggctgccacttgaaagaagaggtatggacgaactatcctagcgatcagtgtgtctattttgcctaacctagcaaagctatatccgcggatctcctggcaaccttcagcctcttcgagcagttcgcagccgcagcatattgtccggataacaacgacagtcccgacaccaagcttacttgctctgtcggaaactgcccgcttgtcgaagctgacacgaccagcacggtcactgaattcgaaaagtacatcttacacgaccccgttcacctacagacaaagtcccagctaacgtccacctctatctctgtccctttagctcgctcgaaaccgacgtcactggctacgtcgcgactgacagcacacgagagctcatcgttgtggcattccgcgggagttcctcgatccggaactggatcgccgacatcgactttcccttcaccgacaccgacctctgcgatggctgccaggcagcctcgggcttctggacgtcctggacggaggcacggacaggggtgctggcggcggtggcgagcgctgccgcggccaacccgtcctataccgttgccgtgacgggccacagcctcggcggggccgtggccgcgctggccgctggcgccctccggaacgcgggctacacggtcgcgctatacagcttcggagcgcctcgcgtgggtgacgagaccctcagcgagtacatcactgcgcaggcgggtggaaactaccgcatcacgcacctcaacgacccagtgccgaagctgcccccgctgctcctggggtatcgccacatcagcccggaatactacatcagcagcgggaacaacgtgaccgtgacggcggatgacgtggaggagtacaccggcacgatcaacctgagtgggaacacgggcgatctgacgttcgacacggatgcgcacagttggtacttcaacgagatcggggcatgcgatgatggtgaggctttggagtggaagaagcggggggtagaagttcagtgggttaaacgagccgctgttgactcgaaccataccccggccgctcctgaacttgttgcccggttgcctttggaaaggagggcgatttccgcagacctcctcgcgaccttctccttgttcgaacagttcgcagcagcagcctactgtcccgacaacaacgactcccctgatactaagttgacatgttcggtcggcaactgtcctttggtcgaagccgacacaacatcgaccgtgacagagttcgagaactccctcgagacagacgtcacgggttatgtggcaaccgattccacgcgtgagctcatcgtcgtcgccttcaggggatcctcgtccatccggaactggattgccgacatcgatttccccttcaccgataccgatctctgtgatggttgtcaggcagcatcgggcttctggacctcgtggacagaagcccgaacaggtgtgctcgcagccgtggcgtccgcagcagcagcgaacccctcctacacggtggcagtgacaggccattcgttgggtggtgcggtcgcagccctcgcagcaggtgccttgaggaacgcaggctacacagtggcgttgtactccttcggtgcacctcgggtcggcgacgagacattgtcggagtatatcactgcgcaggcaggtggcaactacaggattactcacctcaacgacccggtccctaagctccctccgttgctcttgggctatcgacacatttcgcctgagtattacatctcgtccggcaacaacgtcacggtgacagccgatgatgtggaggagtacactggaacaatcaacttgtcgggtaacacaggcgatttgaccttcgacacagacgcccactcgtggtatttcaacgagattggtgcgtgtgatgatggcgaggcattggaatggaagaaacgcggagtcgaagtgcagtgggtctaa

SEQ ID NO: 10 - DNA, 41 bp, Artificial Sequence
  Primer lipVR-C
tacacaactgggggccaccatgaagttcttcaccaccatcc

SEQ ID NO: 11 - DNA, 36 bp, Artificial Sequence
  Primer lipVR-D
gtgtcagtcaccgcgttagacccactgcacttcgac